European Patent Application EP 4 361 137 A1, published May 1, 2024. Title: PRUNE_1 INHIBITORS AND THERAPEUTIC USE THEREOF. Applicant: CEINGE BIOTECNOLOGIE AVANZATE SCARL. The sequence listing filed with the application follows.

SEQUENCE LISTING (60 sequences)

SEQ ID NO: 1 - DNA, 24 bp, synthetic construct
  source 1..24: mol_type = other DNA
gacccagatcatgtttgagacctt

SEQ ID NO: 2 - DNA, 21 bp, synthetic construct
  source 1..21: mol_type = other DNA
ccagaggcgtacagggatagc

SEQ ID NO: 3 - DNA, 23 bp, synthetic construct
  source 1..23: mol_type = other DNA
atgatggcttattacagtggcaa

SEQ ID NO: 4 - DNA, 23 bp, synthetic construct
  source 1..23: mol_type = other DNA
atgatggcttattacagtggcaa

SEQ ID NO: 5 - DNA, 21 bp, synthetic construct
  source 1..21: mol_type = other DNA
tcaggcaggcagtatcactca

SEQ ID NO: 6 - DNA, 20 bp, synthetic construct
  source 1..20: mol_type = other DNA
aggtccacgggaaagacaca

SEQ ID NO: 7 - DNA, 20 bp, synthetic construct
  source 1..20: mol_type = other DNA
cagttctatggcccagaccc

SEQ ID NO: 8 - DNA, 20 bp, synthetic construct
  source 1..20: mol_type = other DNA
acgtgggctacaggcttgtc

SEQ ID NO: 9 - DNA, 20 bp, synthetic construct
  source 1..20: mol_type = other DNA
atcacacgggaccaaaccag

SEQ ID NO: 10 - DNA, 21 bp, synthetic construct
  source 1..21: mol_type = other DNA
ccaggcaactctcgttcttgt

SEQ ID NO: 11 - DNA, 26 bp, synthetic construct
  source 1..26: mol_type = other DNA
cttccagagatacaaagaaatgatgg

SEQ ID NO: 12 - DNA, 24 bp, synthetic construct
  source 1..24: mol_type = other DNA
ctccagaagaccagaggaaatttt

SEQ ID NO: 13 - DNA, 20 bp, synthetic construct
  source 1..20: mol_type = other DNA
ccagtacagccgggaagaca

SEQ ID NO: 14 - DNA, 20 bp, synthetic construct
  source 1..20: mol_type = other DNA
cgcagctctaggagcatgtg

SEQ ID NO: 15 - DNA, 20 bp, synthetic construct
  source 1..20: mol_type = other DNA
aggccaaccgtgaaaagatg

SEQ ID NO: 16 - DNA, 21 bp, synthetic construct
  source 1..21: mol_type = other DNA
gcctggatggctacgtacatg

SEQ ID NO: 17 - DNA, 19 bp, synthetic construct
  source 1..19: mol_type = other DNA
agcatccacgtgttggctc

SEQ ID NO: 18 - DNA, 20 bp, synthetic construct
  source 1..20: mol_type = other DNA
ttgggatcatcttgctggtg

SEQ ID NO: 19 - DNA, 23 bp, synthetic construct
  source 1..23: mol_type = other DNA
tacccgctgtatagctacctcga

SEQ ID NO: 20 - DNA, 23 bp, synthetic construct
  source 1..23: mol_type = other DNA
gccacgaccatacagatactgga

SEQ ID NO: 21 - DNA, 20 bp, synthetic construct
  source 1..20: mol_type = other DNA
tgaagtgcacccgtgaaaca

SEQ ID NO: 22 - DNA, 19 bp, synthetic construct
  source 1..19: mol_type = other DNA
tcttccgagctgctacctc

SEQ ID NO: 23 - DNA, 20 bp, synthetic construct
  source 1..20: mol_type = other DNA
acctccaacctgtttcgcct

SEQ ID NO: 24 - DNA, 22 bp, synthetic construct
  source 1..22: mol_type = other DNA
agggttccaggtcagacacact

SEQ ID NO: 25 - DNA, 20 bp, synthetic construct
  source 1..20: mol_type = other DNA
ctgcagcggacagacctctt

SEQ ID NO: 26 - DNA, 20 bp, synthetic construct
  source 1..20: mol_type = other DNA
gcaaccagggcatcatagct

SEQ ID NO: 27 - DNA, 20 bp, synthetic construct
  source 1..20: mol_type = other DNA
ctggccaactcaccctcatc

SEQ ID NO: 28 - DNA, 20 bp, synthetic construct
  source 1..20: mol_type = other DNA
tgcctcctctagggctgtgt

SEQ ID NO: 29 - DNA, 19 bp, synthetic construct
  source 1..19: mol_type = other DNA
cagcagcaggtgtcccaaa

SEQ ID NO: 30 - DNA, 22 bp, synthetic construct
  source 1..22: mol_type = other DNA
tgtctggacccattccttcttg

SEQ ID NO: 31 - DNA, 20 bp, synthetic construct
  source 1..20: mol_type = other DNA
cagaagaatggaagagtcag

SEQ ID NO: 32 - DNA, 20 bp, synthetic construct
  source 1..20: mol_type = other DNA
cagatatgcagggagtcacc

SEQ ID NO: 33 - DNA, 20 bp, synthetic construct
  source 1..20: mol_type = other DNA
gagccatttccatcctgcag

SEQ ID NO: 34 - DNA, 21 bp, synthetic construct
  source 1..21: mol_type = other DNA
gcctgtggctgaagaaaaagg

SEQ ID NO: 35 - DNA, 19 bp, synthetic construct
  source 1..19: mol_type = other DNA
tgcggtatggacttgctgc

SEQ ID NO: 36 - DNA, 21 bp, synthetic construct
  source 1..21: mol_type = other DNA
gaagatgtctgggtaccgggt

SEQ ID NO: 37 - DNA, 21 bp, synthetic construct
  source 1..21: mol_type = other DNA
taccagccaagcctctaagcc

SEQ ID NO: 38 - DNA, 23 bp, synthetic construct
  source 1..23: mol_type = other DNA
tcaatgatgggcctctgacttca

SEQ ID NO: 39 - DNA, 21 bp, synthetic construct
  source 1..21: mol_type = other DNA
tggtgtggaagaagagcaagg

SEQ ID NO: 40 - DNA, 20 bp, synthetic construct
  source 1..20: mol_type = other DNA
agtgccatgaggtccgagtg

SEQ ID NO: 41 - DNA, 20 bp, synthetic construct
  source 1..20: mol_type = other DNA
cggacccagaatacacgcac

SEQ ID NO: 42 - DNA, 21 bp, synthetic construct
  source 1..21: mol_type = other DNA
caaaagttgctctgcattggc

SEQ ID NO: 43 - DNA, 22 bp, synthetic construct
  source 1..22: mol_type = other DNA
tatgacccagactcacaatgga

SEQ ID NO: 44 - DNA, 21 bp, synthetic construct
  source 1..21: mol_type = other DNA
gtgactctgcattcctcaggc

SEQ ID NO: 45 - DNA, 21 bp, synthetic construct
  source 1..21: mol_type = other DNA
acaagggctcaatgaggagat

SEQ ID NO: 46 - DNA, 22 bp, synthetic construct
  source 1..22: mol_type = other DNA
aaagccagaacgtagaggagga

SEQ ID NO: 47 - DNA, 24 bp, synthetic construct
  source 1..24: mol_type = other DNA
aggatgatggcacacacttctcta

SEQ ID NO: 48 - DNA, 21 bp, synthetic construct
  source 1..21: mol_type = other DNA
ccattggaaagtcctcaacct

SEQ ID NO: 49 - DNA, 18 bp, synthetic construct
  source 1..18: mol_type = other DNA
gaggaggtggctgcttag

SEQ ID NO: 50 - DNA, 15 bp, synthetic construct
  source 1..15: mol_type = other DNA
tctgcaacggtttca

SEQ ID NO: 51 - DNA, 19 bp, synthetic construct
  source 1..19: mol_type = other DNA
cccaaaaaatacccaagag

SEQ ID NO: 52 - DNA, 21 bp, synthetic construct
  source 1..21: mol_type = other DNA
cctttacgcaatttggaaacc

SEQ ID NO: 53 - DNA, 21 bp, synthetic construct
  source 1..21: mol_type = other DNA
tggtaggaaggccaatgtgaa

SEQ ID NO: 54 - DNA, 18 bp, synthetic construct
  source 1..18: mol_type = other DNA
tgaacgccaaaggcaaac

SEQ ID NO: 55 - DNA, 17 bp, synthetic construct
  source 1..17: mol_type = other DNA
gatcgtcgtgcatttgc

SEQ ID NO: 56 - DNA, 21 bp, synthetic construct
  source 1..21: mol_type = other DNA
gagtcgatgggctcctcattt

SEQ ID NO: 57 - DNA, 21 bp, synthetic construct
  source 1..21: mol_type = other DNA
tcctgtgaaacagtatggaag

SEQ ID NO: 58 - DNA, 21 bp, synthetic construct
  source 1..21: mol_type = other DNA
tcttgtagcctcttcaaggag

SEQ ID NO: 59 - DNA, 19 bp, synthetic construct
  source 1..19: mol_type = other DNA
tggagtttgattgctgcca

SEQ ID NO: 60 - DNA, 22 bp, synthetic construct
  source 1..22: mol_type = other DNA
tggcatagattcttggatcagg